European Patent Application EP 4 353 832 A1, published April 17, 2024. Title: METHOD AND KIT FOR DETECTING N6-METHYLADENINE IN NUCLEIC ACID MOLECULES. Applicant: PEKING UNIVERSITY. Application PCT/CN2021/130282. The sequence listing filed with the application follows.

SEQUENCE LISTING (20 sequences)

SEQ ID NO: 1 - DNA, 78 bp, Artificial Sequence
  Sequence of DNA model
  misc_feature (23)..(23): n is N6-methyladenine deoxyribonucleotide
gtgtgttgtgtgtgtttgtgcgngtaactgaccagatctctatacgtgactcatgatggctttggttggttggtttgg

SEQ ID NO: 2 - DNA, 86 bp, Artificial Sequence
  Sequence of DNA amplification primer 1
aactggagagcatcctgctgttggtccacatggctagtgatggctactgagtcaggtccattgatgcaccaaaccaaccaaccaaa

SEQ ID NO: 3 - DNA, 20 bp, Artificial Sequence
  Sequence of DNA amplification primer 2
gtgtgttgtgtgtgtttgtg

SEQ ID NO: 4 - DNA, 20 bp, Artificial Sequence
  Primer for DNA sequencing
aactggagagcatcctgctg

SEQ ID NO: 5 - DNA, 19 bp, Artificial Sequence
  Sequence of 3'RNA linker
agatcggaagagcgtcgtg

SEQ ID NO: 6 - DNA, 32 bp, Artificial Sequence
  Sequence of 5'adaptor
  misc_feature (1)..(10): n is a, c, g, or t
nnnnnnnnnnagatcggaagagcacacgtctg

SEQ ID NO: 7 - DNA, 58 bp, Artificial Sequence
  Sequence of cDNA amplification primer 1
aatgatacggcgaccaccgagatctacactctttccctacacgacgctcttccgatct

SEQ ID NO: 8 - DNA, 63 bp, Artificial Sequence
  Sequence of cDNA amplification primer 2
  misc_feature (25)..(30): n is a, c, g, or t
caagcagaagacggcatacgagatnnnnnngtgactggagttcagacgtgtgctcttccgatc

SEQ ID NO: 9 - RNA, 74 nt, Artificial Sequence
  Nucleotide sequence of Spike in 1
guugaucuuggcacgucuacucgaccgucuggaacuugauauuaucggaucagugaaucacuccaagcugacag

SEQ ID NO: 10 - RNA, 74 nt, Artificial Sequence
  Nucleotide sequence of Spike in 2
  misc_feature (40)..(40): n is N6-methyladenine ribonucleotide
agcgcagcgaacaugacacgugcucaacaguguaguuggncuuccucgcaucuagccgcuaugcacgugcagcu

SEQ ID NO: 11 - RNA, 74 nt, Artificial Sequence
  Nucleotide sequence of Spike in 2'
agcgcagcgaacaugacacgugcucaacaguguaguuggacuuccucgcaucuagccgcuaugcacgugcagcu

SEQ ID NO: 12 - RNA, 75 nt, Artificial Sequence
  Nucleotide sequence of Spike in 3
  misc_feature (39)..(39): n is N6-methyladenine ribonucleotide
gaucguagcauugguuagcguguugguggauguagugancuaaucgccuuauaggugccaaaugucauggacagc

SEQ ID NO: 13 - RNA, 75 nt, Artificial Sequence
  Nucleotide sequence of Spike in 3'
gaucguagcauugguuagcguguugguggauguagugaacuaaucgccuuauaggugccaaaugucauggacagc

SEQ ID NO: 14 - RNA, 74 nt, Artificial Sequence
  Nucleotide sequence of Spike in 4
  misc_feature (48)..(48): n is N6-methyladenine ribonucleotide
aucuaccuguccaguagccuucaggaucaugcugucugacuugcuggncaucauucuagugccauaacuucagc

SEQ ID NO: 15 - RNA, 74 nt, Artificial Sequence
  Nucleotide sequence of Spike in 4'
aucuaccuguccaguagccuucaggaucaugcugucugacuugcuggacaucauucuagugccauaacuucagc

SEQ ID NO: 16 - RNA, 69 nt, Artificial Sequence
  Nucleotide sequence of Spike in 5
  misc_feature (33)..(33): n is N6-methyladenine ribonucleotide
uaugguuuagauugaauguuguuguugugaggnccuuauguaaguugaaugguaauaggaagaaguuug

SEQ ID NO: 17 - RNA, 69 nt, Artificial Sequence
  Nucleotide sequence of Spike in 5'
uaugguuuagauugaauguuguuguugugaggaccuuauguaaguugaaugguaauaggaagaaguuug

SEQ ID NO: 18 - RNA, 71 nt, Artificial Sequence
  Nucleotide sequence of Spike in 6
  misc_feature (30)..(30): n is N6-methyladenine ribonucleotide
uuguuugauggagggggauaauuauuggancagguaguuaauauuguauaauguuguaagauuaaagaggg

SEQ ID NO: 19 - RNA, 71 nt, Artificial Sequence
  Nucleotide sequence of Spike in 6'
uuguuugauggagggggauaauuauuggaacagguaguuaauauuguauaauguuguaagauuaaagaggg

SEQ ID NO: 20 - RNA, 71 nt, Artificial Sequence
  Nucleotide sequence of Spike in 7
  misc_feature (34)..(34): n is N6-methyladenine ribonucleotide
ggauuaguuaguaggugggguaaugguuuauganccugaugauuuuuaguugguuugagaggaugauuagu